European Patent Application EP 4 806 920 A1, published September 16, 2026. Title: CD38 antibodies and fragments thereof. Applicant: Georg-August-Universität Göttingen Stiftung Öffentlichen Rechts. The sequence listing filed with the application follows.

SEQUENCE LISTING (77 sequences)

SEQ ID NO: 1 - DNA, 366 bp, synthetic construct
  source 1..366: mol_type = other DNA
gaggtgcagctggtggagtctgggggaggcttggtgcaggctggggggtctctgagactctcctgtgcagtctctggaggcgcgttcaataactttgccatgggctggttccgccaggctccagggaaggagcgtgagtttgttgcagctattacctggggttctggcacactctatgcagactccgtgaagggccgattcaccctctccagagacaaccccaaaaacacggcgtatctgcaaatggacagtctgaaacctgaggacacggccgtttatttctgtgcaggaaagtatttcacgacggcccgactaccggcggaatataagtactggggtcaggggacccaggtcaccgtctcctca

SEQ ID NO: 2 - protein, 122 aa, synthetic construct
EVQLVESGGGLVQAGGSLRLSCAVSGGAFNNFAMGWFRQAPGKEREFVAAITWGSGTLYADSVKGRFTLSRDNPKNTAYLQMDSLKPEDTAVYFCAGKYFTTARLPAEYKYWGQGTQVTVSS

SEQ ID NO: 3 - protein, 26 aa, synthetic construct
EVQLVESGGGLVQAGGSLRLSCAVSG

SEQ ID NO: 4 - protein, 6 aa, synthetic construct
GAFNNF

SEQ ID NO: 5 - protein, 19 aa, synthetic construct
AMGWFRQAPGKEREFVAAI

SEQ ID NO: 6 - protein, 6 aa, synthetic construct
TWGSGT

SEQ ID NO: 7 - protein, 40 aa, synthetic construct
LYADSVKGRFTLSRDNPKNTAYLQMDSLKPEDTAVYFCAG

SEQ ID NO: 8 - protein, 14 aa, synthetic construct
KYFTTARLPAEYKY

SEQ ID NO: 9 - protein, 11 aa, synthetic construct
WGQGTQVTVSS

SEQ ID NO: 10 - DNA, 375 bp, synthetic construct
  source 1..375: mol_type = other DNA
gaggtgcagctggaggagtctgggggaggattggtgcaggctgggggctcgctaagactctcctgtgcagcctctggacgcaccctcagtaactatcacatgggctggttccgccaggctccagggaaggagcgtgagtttgtagcagctattaactggagcggtcttaacacatactatatggactccgtgaagggccgattcaccgtctccagagacaacgccaagaacacggtgtatctgcaaatgaacagcctgaaacctgaggacacggccgtttattactgtgcagcacaattcttcgcggcagcagttggtagggactctgcgaagtatgcgtactggggccaggggacccaggtcaccgtctcctca

SEQ ID NO: 11 - protein, 125 aa, synthetic construct
EVQLEESGGGLVQAGGSLRLSCAASGRTLSNYHMGWFRQAPGKEREFVAAINWSGLNTYYMDSVKGRFTVSRDNAKNTVYLQMNSLKPEDTAVYYCAAQFFAAAVGRDSAKYAYWGQGTQVTVSS

SEQ ID NO: 12 - protein, 26 aa, synthetic construct
EVQLEESGGGLVQAGGSLRLSCAASG

SEQ ID NO: 13 - protein, 7 aa, synthetic construct
RTLSNYH

SEQ ID NO: 14 - protein, 18 aa, synthetic construct
MGWFRQAPGKEREFVAAI

SEQ ID NO: 15 - protein, 6 aa, synthetic construct
NWSGLN

SEQ ID NO: 16 - protein, 41 aa, synthetic construct
TYYMDSVKGRFTVSRDNAKNTVYLQMNSLKPEDTAVYYCAA

SEQ ID NO: 17 - protein, 16 aa, synthetic construct
QFFAAAVGRDSAKYAY

SEQ ID NO: 18 - protein, 11 aa, synthetic construct
WGQGTQVTVSS

SEQ ID NO: 19 - DNA, 369 bp, synthetic construct
  source 1..369: mol_type = other DNA
gaggtgcagctgctggagtctgggggaggattggtgcaggctggggcctctctgagactctcctgtgcagcctctggacgcaccttcagaaactctgccatgggctggttctgccaggctccagggaaggggcgtgagtttgtagcaggcatgagctggagtggcagcacactctatgcagactccgtgaagggccgattcactatctccagagacaacgccaagaacatggtgtatctgcaaatgaacagcctggcacctgaggacacggccgtttatttctgtgcagcaaggagccgtatgtttgtaaccagatcaccggacgagtatgactactggggccaggggacccaggtcaccgtctcctca

SEQ ID NO: 20 - protein, 123 aa, synthetic construct
EVQLLESGGGLVQAGASLRLSCAASGRTFRNSAMGWFCQAPGKGREFVAGMSWSGSTLYADSVKGRFTISRDNAKNMVYLQMNSLAPEDTAVYFCAARSRMFVTRSPDEYDYWGQGTQVTVSS

SEQ ID NO: 21 - protein, 26 aa, synthetic construct
EVQLLESGGGLVQAGASLRLSCAASG

SEQ ID NO: 22 - protein, 7 aa, synthetic construct
RTFRNSA

SEQ ID NO: 23 - protein, 18 aa, synthetic construct
MGWFCQAPGKGREFVAGM

SEQ ID NO: 24 - protein, 6 aa, synthetic construct
SWSGST

SEQ ID NO: 25 - protein, 40 aa, synthetic construct
LYADSVKGRFTISRDNAKNMVYLQMNSLAPEDTAVYFCAA

SEQ ID NO: 26 - protein, 15 aa, synthetic construct
RSRMFVTRSPDEYDY

SEQ ID NO: 27 - protein, 11 aa, synthetic construct
WGQGTQVTVSS

SEQ ID NO: 28 - DNA, 375 bp, synthetic construct
  source 1..375: mol_type = other DNA
gaggtgcagctggaggagtctgggggaggattggtgcaggctgggggctctctaagactctcctgtgcagcctccgaacgcaccttcggtaactaccccatgggctggttccgccaggttccagggaaggaacgtgagtttgtagcagctattactgggcttgcgggtagccgactctatgcagactccgcgaagggccgcttcaccatctcccgagacaacgccaagaacacggtgtatctgcaaatgaacaacctacaacctgaggacacgggcgtttattactgtgcagcggatcgacgaataggtggagtaacgagggagtcgagggagtacgagtactggggtcaggggacccaggtcaccgtctcctca

SEQ ID NO: 29 - protein, 125 aa, synthetic construct
EVQLEESGGGLVQAGGSLRLSCAASERTFGNYPMGWFRQVPGKEREFVAAITGLAGSRLYADSAKGRFTISRDNAKNTVYLQMNNLQPEDTGVYYCAADRRIGGVTRESREYEYWGQGTQVTVSS

SEQ ID NO: 30 - protein, 26 aa, synthetic construct
EVQLEESGGGLVQAGGSLRLSCAASE

SEQ ID NO: 31 - protein, 7 aa, synthetic construct
RTFGNYP

SEQ ID NO: 32 - protein, 18 aa, synthetic construct
MGWFRQVPGKEREFVAAI

SEQ ID NO: 33 - protein, 6 aa, synthetic construct
TGLAGS

SEQ ID NO: 34 - protein, 41 aa, synthetic construct
RLYADSAKGRFTISRDNAKNTVYLQMNNLQPEDTGVYYCAA

SEQ ID NO: 35 - protein, 16 aa, synthetic construct
DRRIGGVTRESREYEY

SEQ ID NO: 36 - protein, 11 aa, synthetic construct
WGQGTQVTVSS

SEQ ID NO: 37 - DNA, 378 bp, synthetic construct
  source 1..378: mol_type = other DNA
gaggtgcagctgctggagtctgggggaggattggtgcaggctggggactctctgcgactctcctgtgtagcctctggacgtacttctagtttctataccatggcctggttccgccaggctccagggaaggagcgtgagtttgtagcgtcggttgggtggagtggtggaagcacattatatgctgactccgtgaagggccgaagcaccatctccagagacaacgccaacgccaagaatatgttgtatttgcaagtggacaggctgaaagttgaggacacggccgtttattactgtgcaaccagaaggggcgtcagtagttcgcggttggtcagtgagtatgactactggggccaggggacccaggtcaccgtctcctca

SEQ ID NO: 38 - protein, 126 aa, synthetic construct
EVQLLESGGGLVQAGDSLRLSCVASGRTSSFYTMAWFRQAPGKEREFVASVGWSGGSTLYADSVKGRSTISRDNANAKNMLYLQVDRLKVEDTAVYYCATRRGVSSSRLVSEYDYWGQGTQVTVSS

SEQ ID NO: 39 - protein, 26 aa, synthetic construct
EVQLLESGGGLVQAGDSLRLSCVASG

SEQ ID NO: 40 - protein, 7 aa, synthetic construct
RTSSFYT

SEQ ID NO: 41 - protein, 18 aa, synthetic construct
MAWFRQAPGKEREFVASV

SEQ ID NO: 42 - protein, 6 aa, synthetic construct
GWSGGS

SEQ ID NO: 43 - protein, 43 aa, synthetic construct
TLYADSVKGRSTISRDNANAKNMLYLQVDRLKVEDTAVYYCAT

SEQ ID NO: 44 - protein, 15 aa, synthetic construct
RRGVSSSRLVSEYDY

SEQ ID NO: 45 - protein, 11 aa, synthetic construct
WGQGTQVTVSS

SEQ ID NO: 46 - DNA, 396 bp, synthetic construct
  source 1..396: mol_type = other DNA
gaggtgcagctgctggagtctgggggaggattggtgcaggctggggcctctctgagactctcatgtgcaacttctggacgcacactcagtaactttgccatgggctggttccgccaggctccaggtaaggggcgtgagtttgtagcagctgtgagctgggctgcaagcacactctatgcggactccgtgaagggccgattcaccatctccagagacaacgccaaaaacatgctgtatctccaaatgaacagcctgaaacctgaggacacggccgtatatttttgtgcagcaaggaagcgtatgtgggtagacagatcaccggatgagtataactactggggccaggggacccaggtcaccgtctcctcagaacccaagaaaccaaaaccacaaact

SEQ ID NO: 47 - protein, 132 aa, synthetic construct
EVQLLESGGGLVQAGASLRLSCATSGRTLSNFAMGWFRQAPGKGREFVAAVSWAASTLYADSVKGRFTISRDNAKNMLYLQMNSLKPEDTAVYFCAARKRMWVDRSPDEYNYWGQGTQVTVSSEPKKPKPQT

SEQ ID NO: 48 - DNA, 366 bp, synthetic construct
  source 1..366: mol_type = other DNA
gaggtgcagctggtggagtctgggggaggattggtgcaggctgggggctctctgagactctcctgtgcagtctctggaggcacgttcaataactttgccatgggctggttccgccaggctccaggggaggagcgtgagtttgttgcagctattacctggggttctggcacactctatgcagactccgtgaagggccgattcatcctctccagaaacaacgccaaaaacacggcgtatctgcaaatgaacagcctgaaacctgaggacacggccgtttattactgtgcaggaaagtatttcacggttgacagactaccaaccgagtacaagtactggggccaggggacccaggtcaccgtctcctca

SEQ ID NO: 49 - protein, 122 aa, synthetic construct
EVQLVESGGGLVQAGGSLRLSCAVSGGTFNNFAMGWFRQAPGEEREFVAAITWGSGTLYADSVKGRFILSRNNAKNTAYLQMNSLKPEDTAVYYCAGKYFTVDRLPTEYKYWGQGTQVTVSS

SEQ ID NO: 50 - protein, 26 aa, synthetic construct
EVQLVESGGGLVQAGGSLRLSCAVSG

SEQ ID NO: 51 - protein, 6 aa, synthetic construct
GTFNNF

SEQ ID NO: 52 - protein, 18 aa, synthetic construct
MAWFRQAPGKEREFVASV

SEQ ID NO: 53 - protein, 6 aa, synthetic construct
TWGSGT

SEQ ID NO: 54 - protein, 40 aa, synthetic construct
LYADSVKGRFILSRNNAKNTAYLQMNSLKPEDTAVYYCAG

SEQ ID NO: 55 - protein, 14 aa, synthetic construct
KYFTVDRLPTEYKY

SEQ ID NO: 56 - protein, 11 aa, synthetic construct
WGQGTQVTVSS

SEQ ID NO: 57 - DNA, 372 bp, synthetic construct
  source 1..372: mol_type = other DNA
gaggtgcagctgctggagtctgggggaggattggtgcaggctgggggctctctgagactctcctgtgcagcctctggacgtacttctacattctttaccatggcctggttccgccaggctccagggaaggagcgtgagtttgtagcagcggttgggtggagtggtggtagtacattatatggtgactccgtgaagggccgaagcaccatctccagagacaacgccaagaacacactgtatttgcaagtggacaggctgaaagttgaggacacggccgattattactgcgcaagtaggaggggcgtcagtatttcgcggttggtcagtgagtatgactactggggccaggggacccaggtcaccgtctcctca

SEQ ID NO: 58 - protein, 124 aa, synthetic construct
EVQLLESGGGLVQAGGSLRLSCAASGRTSTFFTMAWFRQAPGKEREFVAAVGWSGGSTLYGDSVKGRSTISRDNAKNTLYLQVDRLKVEDTADYYCASRRGVSISRLVSEYDYWGQGTQVTVSS

SEQ ID NO: 59 - protein, 26 aa, synthetic construct
EVQLLESGGGLVQAGGSLRLSCAASG

SEQ ID NO: 60 - protein, 6 aa, synthetic construct
RTSTFF

SEQ ID NO: 61 - protein, 19 aa, synthetic construct
TMAWFRQAPGKEREFVAAV

SEQ ID NO: 62 - protein, 6 aa, synthetic construct
GWSGGS

SEQ ID NO: 63 - protein, 41 aa, synthetic construct
TLYGDSVKGRSTISRDNAKNTLYLQVDRLKVEDTADYYCAS

SEQ ID NO: 64 - protein, 15 aa, synthetic construct
RRGVSISRLVSEYDY

SEQ ID NO: 65 - protein, 11 aa, synthetic construct
WGQGTQVTVSS

SEQ ID NO: 66 - DNA, 414 bp, synthetic construct
  source 1..414: mol_type = other DNA
gaggtgcagctgctggagtctgggggaggattggtgcaggctgggggctctctgagactctcctgtgtagcctctgaacgcaccgcctctggacgcgccgcctatgtcatgggctggttccgccaggccccggggaaggagcgtgagtttgtgtcagccattaggtggagtgacgatagtacatcgtatgcagactccgtgaagggcagattcaccgtctccagagacaatgccaggaacatggtgtacctgcaaatgaatactgtgaaacctgaggacacggccaattattactgtgcagctcgctttcgatttactataactcctataaccagttcgcgtgactatgactactggggccaggggacccaggtcaccgtctcctcagaacccaagacaccaaaaccacaaact

SEQ ID NO: 67 - protein, 138 aa, synthetic construct
EVQLLESGGGLVQAGGSLRLSCVASERTASGRAAYVMGWFRQAPGKEREFVSAIRWSDDSTSYADSVKGRFTVSRDNARNMVYLQMNTVKPEDTANYYCAARFRFTITPITSSRDYDYWGQGTQVTVSSEPKTPKPQT

SEQ ID NO: 68 - DNA, 366 bp, synthetic construct
  source 1..366: mol_type = other DNA
gaggtgcagctggaggagtctgggggaggattggtgcaggctgggggctctctgagactctcctgtgtagtctctggaggcgcgttcaataactttgccatgggctggttccgccaggctccagggaaggagcgtgagtttgttgcaggcatgagctggagtggcagcacactctatgcagactccgtgaagggccgattcaccctctccagagacaaccccaaaaacacggcgtatctgcaaatggacagtctgaaacctgaggacacggccgtttatttctgtgcaggaaagtatttcacgacggcccgactaccggcggagtataagtactggggtcaggggacccaggtcaccgtctcctca

SEQ ID NO: 69 - protein, 122 aa, synthetic construct
EVQLEESGGGLVQAGGSLRLSCVVSGGAFNNFAMGWFRQAPGKEREFVAGMSWSGSTLYADSVKGRFTLSRDNPKNTAYLQMDSLKPEDTAVYFCAGKYFTTARLPAEYKYWGQGTQVTVSS

SEQ ID NO: 70 - protein, 26 aa, synthetic construct
EVQLEESGGGLVQAGGSLRLSCVVSG

SEQ ID NO: 71 - protein, 7 aa, synthetic construct
GAFNNFA

SEQ ID NO: 72 - protein, 18 aa, synthetic construct
MGWFRQAPGKEREFVAGM

SEQ ID NO: 73 - protein, 6 aa, synthetic construct
SWSGST

SEQ ID NO: 74 - protein, 39 aa, synthetic construct
LYADSVKGRFTLSRDNPKNTAYLQMDSLKPEDTAVYFCA

SEQ ID NO: 75 - protein, 14 aa, synthetic construct
KYFTTARLPAEYKY

SEQ ID NO: 76 - protein, 11 aa, synthetic construct
WGQGTQVTVSS

SEQ ID NO: 77 - protein, 300 aa, Homo sapiens
MANCEFSPVSGDKPCCRLSRRAQLCLGVSILVLILVVVLAVVVPRWRQQWSGPGTTKRFPETVLARCVKYTEIHPEMRHVDCQSVWDAFKGAFISKHPCNITEEDYQPLMKLGTQTVPCNKILLWSRIKDLAHQFTQVQRDMFTLEDTLLGYLADDLTWCGEFNTSKINYQSCPDWRKDCSNNPVSVFWKTVSRRFAEAACDVVHVMLNGSRSKIFDKNSTFGSVEVHNLQPEKVQTLEAWVIHGGREDSRDLCQDPTIKELESIISKRNIQFSCKNIYRPDKFLQCVKNPEDSSCTSEI